European Patent Application EP 4 449 858 A2, published October 23, 2024. Title: COMPOSITIONS AND METHODS FOR ENHANCING RESISTANCE TO NORTHERN LEAF BLIGHT IN MAIZE. Applicant: Corteva Agriscience LLC. Application EP. The sequence listing filed with the application follows.

SEQUENCE LISTING (97 sequences)

SEQ ID NO: 1 - DNA, 20 bp, synthetic construct
  misc_feature 1..20: note = PHM2798 F Primer
  source 1..20: mol_type = other DNA
gactcggttaagaagaggga

SEQ ID NO: 2 - DNA, 20 bp, synthetic construct
  misc_feature 1..20: note = PHM2798 R Primer
  source 1..20: mol_type = other DNA
tcaagaatcctaggtggcag

SEQ ID NO: 3 - DNA, 20 bp, synthetic construct
  misc_feature 1..20: note = b0302H1 F primer
  source 1..20: mol_type = other DNA
tatgggagaagatggcaacc

SEQ ID NO: 4 - DNA, 20 bp, synthetic construct
  misc_feature 1..20: note = b0302H1 R Primer
  source 1..20: mol_type = other DNA
cccacttaagggttgtgtcc

SEQ ID NO: 5 - DNA, 20 bp, synthetic construct
  misc_feature 1..20: note = b0611n13 F Primer
  source 1..20: mol_type = other DNA
ttgttgggcttcgtatctcc

SEQ ID NO: 6 - DNA, 19 bp, synthetic construct
  misc_feature 1..19: note = b0611n13 R Primer
  source 1..19: mol_type = other DNA
catgcctcaaattgcaagg

SEQ ID NO: 7 - DNA, 20 bp, synthetic construct
  misc_feature 1..20: note = 2717_3 F Primer
  source 1..20: mol_type = other DNA
ggcgactacagggttagagc

SEQ ID NO: 8 - DNA, 20 bp, synthetic construct
  misc_feature 1..20: note = 2717_3 R Primer
  source 1..20: mol_type = other DNA
ggccttccatatcagtttcg

SEQ ID NO: 9 - DNA, 20 bp, synthetic construct
  misc_feature 1..20: note = 2717_4 F Primer
  source 1..20: mol_type = other DNA
actcctgctcctcttgttcg

SEQ ID NO: 10 - DNA, 20 bp, synthetic construct
  misc_feature 1..20: note = 2717_4 R Primer
  source 1..20: mol_type = other DNA
cgctacccgttctatcttgc

SEQ ID NO: 11 - DNA, 21 bp, synthetic construct
  misc_feature 1..21: note = 108f16_2 F Primer
  source 1..21: mol_type = other DNA
gagtgggtgtcgtagttcagc

SEQ ID NO: 12 - DNA, 20 bp, synthetic construct
  misc_feature 1..20: note = 108f16_2 R Primer
  source 1..20: mol_type = other DNA
tcgactacaagacgcgtacc

SEQ ID NO: 13 - DNA, 20 bp, synthetic construct
  misc_feature 1..20: note = 31004 F Primer
  source 1..20: mol_type = other DNA
ctcaccggtccttcacaatg

SEQ ID NO: 14 - DNA, 19 bp, synthetic construct
  misc_feature 1..19: note = 31004 R Primer
  source 1..19: mol_type = other DNA
caaggcgcacgttagacac

SEQ ID NO: 15 - DNA, 21 bp, synthetic construct
  misc_feature 1..21: note = pco642297_3 F Primer
  source 1..21: mol_type = other DNA
cgaccgacgatagatggtgtc

SEQ ID NO: 16 - DNA, 24 bp, synthetic construct
  misc_feature 1..24: note = pco642297_3 R Primer
  source 1..24: mol_type = other DNA
atgttgctccaacagatactttgc

SEQ ID NO: 17 - DNA, 23 bp, synthetic construct
  misc_feature 1..23: note = b109.m6 F Primer
  source 1..23: mol_type = other DNA
gctgagttggatatggtctatgg

SEQ ID NO: 18 - DNA, 20 bp, synthetic construct
  misc_feature 1..20: note = b109.m6 R Primer
  source 1..20: mol_type = other DNA
ttcaggtgctaggtttgtgg

SEQ ID NO: 19 - DNA, 19 bp, synthetic construct
  misc_feature 1..19: note = PHM18979 F Primer
  source 1..19: mol_type = other DNA
ggtcaatcggactacagtg

SEQ ID NO: 20 - DNA, 20 bp, synthetic construct
  misc_feature 1..20: note = PHM18979 R Primer
  source 1..20: mol_type = other DNA
aaagcagggttagtgcgact

SEQ ID NO: 21 - DNA, 20 bp, synthetic construct
  misc_feature 1..20: note = b0507L21 F Primer
  source 1..20: mol_type = other DNA
agcaccacacaggagacacg

SEQ ID NO: 22 - DNA, 19 bp, synthetic construct
  misc_feature 1..19: note = b0507L21 R Primer
  source 1..19: mol_type = other DNA
gtgcctggagatgttgacg

SEQ ID NO: 23 - DNA, 20 bp, synthetic construct
  misc_feature 1..20: note = 2_2 F Primer
  source 1..20: mol_type = other DNA
gagacatggtgtttgcatgg

SEQ ID NO: 24 - DNA, 20 bp, synthetic construct
  misc_feature 1..20: note = 2_2 R Primer
  source 1..20: mol_type = other DNA
ttcttgggctctctctaccg

SEQ ID NO: 25 - DNA, 19 bp, synthetic construct
  misc_feature 1..19: note = 156k16 F Primer
  source 1..19: mol_type = other DNA
agtgcacttggcaacaagc

SEQ ID NO: 26 - DNA, 20 bp, synthetic construct
  misc_feature 1..20: note = 156k16 R Primer
  source 1..20: mol_type = other DNA
catgtccaggacctttaccg

SEQ ID NO: 27 - DNA, 22 bp, synthetic construct
  misc_feature 1..22: note = b0318i13 F Primer
  source 1..22: mol_type = other DNA
gatcaagatgggaattctttcg

SEQ ID NO: 28 - DNA, 20 bp, synthetic construct
  misc_feature 1..20: note = b0318i13 R Primer
  source 1..20: mol_type = other DNA
ttccacatccaacatcaagc

SEQ ID NO: 29 - DNA, 19 bp, synthetic construct
  misc_feature 1..19: note = PHM4757 F Primer
  source 1..19: mol_type = other DNA
tcctgaacgcgagcctcta

SEQ ID NO: 30 - DNA, 21 bp, synthetic construct
  misc_feature 1..21: note = PHM4757 R Primer
  source 1..21: mol_type = other DNA
taacgagtctcgtctccagaa

SEQ ID NO: 31 - DNA, 23 bp, synthetic construct
  misc_feature 1..23: note = NLB5A F Primer
  source 1..23: mol_type = other DNA
gctgaactagtagcacggcatgt

SEQ ID NO: 32 - DNA, 22 bp, synthetic construct
  misc_feature 1..22: note = NLB5A R Primer
  source 1..22: mol_type = other DNA
agcggagagacggatagagaga

SEQ ID NO: 33 - DNA, 255 bp, synthetic construct
  misc_feature 1..255: note = NLB5A probe
  misc_feature 78..94: note = n is a, c, g, or t
  source 1..255: mol_type = other DNA
gctgaactagtagcacggcatgtactgtcgccgccagtccaggtccaggcgtccagcgaggcagcagcaaacgcagcnnnnnnnnnnnnnnnnncccgcctcagccgatccgagacattcctgtctgggtgagggtgaggccaaccaaccgcttcgctcctctcggtaaatcggcgatccatccagcggagccgcaaccaaaaagcagagcaacgcccaaattaaaaacagggcaggggaaaaaaaaagctcgca

SEQ ID NO: 34 - DNA, 22 bp, synthetic construct
  misc_feature 1..22: note = NLB3A F Primer
  source 1..22: mol_type = other DNA
ggtgtccgcacactcttcttct

SEQ ID NO: 35 - DNA, 22 bp, synthetic construct
  misc_feature 1..22: note = NLB3A R Primer
  source 1..22: mol_type = other DNA
aaagcaaattgaacgcacgagt

SEQ ID NO: 36 - DNA, 255 bp, synthetic construct
  misc_feature 1..255: note = NLB3A probe
  misc_feature 122..139: note = n is a, c, g, or t
  misc_feature 248..255: note = n is a, c, g, or t
  source 1..255: mol_type = other DNA
ggtgtccgcacactcttcttctattgtttgtctactcactccactcccgtcctcgctccttccacgaaactacgttcactagctcgggatgaacagagtcgcctctctctctgctagtcagnnnnnnnnnnnnnnnnnnacacggatcagtttgtaattaccgtgacttcattgccacagctacacaattgcacgagtcaaagtcttttggctggctcctagcacccacacaaaacaacctcgcccgnnnnnnnn

SEQ ID NO: 37 - DNA, 22 bp, synthetic construct
  misc_feature 1..22: note = PHM2817-26 F Primer
  source 1..22: mol_type = other DNA
atatttacagtttcggagtggt

SEQ ID NO: 38 - DNA, 22 bp, synthetic construct
  misc_feature 1..22: note = PHM2817-26 R Primer
  source 1..22: mol_type = other DNA
atctgtgctgataaaaaaaagc

SEQ ID NO: 39 - DNA, 20 bp, synthetic construct
  misc_feature 1..20: note = PHM7446-6 F Primer
  source 1..20: mol_type = other DNA
tggcttacagctgctctgct

SEQ ID NO: 40 - DNA, 22 bp, synthetic construct
  misc_feature 1..22: note = PHM7446-6 R Primer
  source 1..22: mol_type = other DNA
cttggacaaattctgatgattg

SEQ ID NO: 41 - DNA, 20 bp, synthetic construct
  misc_feature 1..20: note = PHM4582 F Primer
  source 1..20: mol_type = other DNA
agtagcctgagtacaatgcc

SEQ ID NO: 42 - DNA, 20 bp, synthetic construct
  misc_feature 1..20: note = PHM4582 R Primer
  source 1..20: mol_type = other DNA
atctctgcacaccatggcaa

SEQ ID NO: 43 - DNA, 23 bp, synthetic construct
  misc_feature 1..23: note = 9g13-3 F primer
  source 1..23: mol_type = other DNA
tcaatctcccaataagctactcg

SEQ ID NO: 44 - DNA, 21 bp, synthetic construct
  misc_feature 1..21: note = 9g13-3 R Primer
  source 1..21: mol_type = other DNA
caagaatgaagcaggtgaagg

SEQ ID NO: 45 - DNA, 18 bp, synthetic construct
  misc_feature 1..18: note = K F Primer
  source 1..18: mol_type = other DNA
tgtagacggtgccgaagc

SEQ ID NO: 46 - DNA, 21 bp, synthetic construct
  misc_feature 1..21: note = K R Primer
  source 1..21: mol_type = other DNA
ctgcaaacacgattagtcagg

SEQ ID NO: 47 - DNA, 20 bp, synthetic construct
  misc_feature 1..20: note = 6_7 F Primer
  source 1..20: mol_type = other DNA
gggctagctgaagctactgg

SEQ ID NO: 48 - DNA, 20 bp, synthetic construct
  misc_feature 1..20: note = 6_7 R Primer
  source 1..20: mol_type = other DNA
tcaccttcttcttcggatgc

SEQ ID NO: 49 - DNA, 20 bp, synthetic construct
  misc_feature 1..20: note = 6_8 F Primer
  source 1..20: mol_type = other DNA
ctccgagcacatctctgtcc

SEQ ID NO: 50 - DNA, 20 bp, synthetic construct
  misc_feature 1..20: note = 6_8 R Primer
  source 1..20: mol_type = other DNA
aaaccgggtcaaagtctacg

SEQ ID NO: 51 - DNA, 20 bp, synthetic construct
  misc_feature 1..20: note = N F Primer
  source 1..20: mol_type = other DNA
acgagctctgtggtttcacc

SEQ ID NO: 52 - DNA, 20 bp, synthetic construct
  misc_feature 1..20: note = N R Primer
  source 1..20: mol_type = other DNA
tcgaaaggtatgccttcacc

SEQ ID NO: 53 - DNA, 20 bp, synthetic construct
  misc_feature 1..20: note = R F Primer
  source 1..20: mol_type = other DNA
aaccagaagaaatggcatgg

SEQ ID NO: 54 - DNA, 21 bp, synthetic construct
  misc_feature 1..21: note = R R Primer
  source 1..21: mol_type = other DNA
tctgtgctatttgtcggaagg

SEQ ID NO: 55 - DNA, 20 bp, synthetic construct
  misc_feature 1..20: note = S F Primer
  source 1..20: mol_type = other DNA
ggttgcttgatgtgcttacg

SEQ ID NO: 56 - DNA, 18 bp, synthetic construct
  misc_feature 1..18: note = S R Primer
  source 1..18: mol_type = other DNA
gcattgcctcttgagtcc

SEQ ID NO: 57 - DNA, 20 bp, synthetic construct
  misc_feature 1..20: note = U F Primer
  source 1..20: mol_type = other DNA
ccgtcctgagcaacattacc

SEQ ID NO: 58 - DNA, 20 bp, synthetic construct
  misc_feature 1..20: note = U R Primer
  source 1..20: mol_type = other DNA
ggagatcaacgaacgagacg

SEQ ID NO: 59 - DNA, 18 bp, synthetic construct
  misc_feature 1..18: note = PHM13395-16 F Primer
  source 1..18: mol_type = other DNA
tccggcgggtccgcggtg

SEQ ID NO: 60 - DNA, 22 bp, synthetic construct
  misc_feature 1..22: note = PHM13395-16 R Primer
  source 1..22: mol_type = other DNA
agacacggttacttctaacgaa

SEQ ID NO: 61 - DNA, 22 bp, synthetic construct
  misc_feature 1..22: note = PHM34318-12 F Primer
  source 1..22: mol_type = other DNA
gatggaagatgctacatatcta

SEQ ID NO: 62 - DNA, 22 bp, synthetic construct
  misc_feature 1..22: note = PHM3418-12 R Primer
  source 1..22: mol_type = other DNA
agcaaaacaaaatccattatta

SEQ ID NO: 63 - DNA, 18 bp, synthetic construct
  misc_feature 1..18: note = PHM13395-27 F Primer
  source 1..18: mol_type = other DNA
tccggcgggtccgcggtg

SEQ ID NO: 64 - DNA, 22 bp, synthetic construct
  misc_feature 1..22: note = PHM13395-27 R Primer
  source 1..22: mol_type = other DNA
agacacggttacttctaacgaa

SEQ ID NO: 65 - DNA, 21 bp, synthetic construct
  misc_feature 1..21: note = PHM4677-11 F Primer
  source 1..21: mol_type = other DNA
agaagaactagagcaacagca

SEQ ID NO: 66 - DNA, 22 bp, synthetic construct
  misc_feature 1..22: note = PHM4677-11 R Primer
  source 1..22: mol_type = other DNA
aatctcaactcaacctccataa

SEQ ID NO: 67 - DNA, 20 bp, synthetic construct
  misc_feature 1..20: note = PHM15992-3 F Primer
  source 1..20: mol_type = other DNA
tataccggcaacattgggag

SEQ ID NO: 68 - DNA, 22 bp, synthetic construct
  misc_feature 1..22: note = PHM15992-3 R Primer
  source 1..22: mol_type = other DNA
gcatttctttacactgcaacaa

SEQ ID NO: 69 - DNA, 23 bp, synthetic construct
  misc_feature 1..23: note = NLB17_A F Primer
  source 1..23: mol_type = other DNA
gtttgttcttcgatttgaaggga

SEQ ID NO: 70 - DNA, 23 bp, synthetic construct
  misc_feature 1..23: note = NLB17_A R Primer
  source 1..23: mol_type = other DNA
accgttttcgaggtaaaatgaag

SEQ ID NO: 71 - DNA, 21 bp, synthetic construct
  misc_feature 1..21: note = NLB17_E F Primer
  source 1..21: mol_type = other DNA
ttcctcacgagctctgtggtt

SEQ ID NO: 72 - DNA, 20 bp, synthetic construct
  misc_feature 1..20: note = NLB17_E R Primer
  source 1..20: mol_type = other DNA
catgctgactagtggtgcgc

SEQ ID NO: 73 - DNA, 26 bp, synthetic construct
  misc_feature 1..26: note = NLB17_3 F Primer
  source 1..26: mol_type = other DNA
caagtaggcttcttgtatccaaattc

SEQ ID NO: 74 - DNA, 22 bp, synthetic construct
  misc_feature 1..22: note = NLB17_3 R Primer
  source 1..22: mol_type = other DNA
gccgagtcgaaacaagttgagt

SEQ ID NO: 75 - DNA, 21 bp, synthetic construct
  misc_feature 1..21: note = NLB18_A F Primer
  source 1..21: mol_type = other DNA
ttgttcttcgatttgaagggc

SEQ ID NO: 76 - DNA, 23 bp, synthetic construct
  misc_feature 1..23: note = NLB18_A R Primer
  source 1..23: mol_type = other DNA
accgttttcgaggtaaaatgaac

SEQ ID NO: 77 - DNA, 21 bp, synthetic construct
  misc_feature 1..21: note = NLB18_E F Primer
  source 1..21: mol_type = other DNA
ttcctcacgagctctgtggtc

SEQ ID NO: 78 - DNA, 25 bp, synthetic construct
  misc_feature 1..25: note = NLB18_E R Primer
  source 1..25: mol_type = other DNA
gtttacatgctgactagtggtgcat

SEQ ID NO: 79 - DNA, 19 bp, synthetic construct
  misc_feature 1..19: note = Sequencing tail added to F primers
  source 1..19: mol_type = other DNA
ggaaacagctatgaccatg

SEQ ID NO: 80 - DNA, 18 bp, synthetic construct
  misc_feature 1..18: note = Sequencing tail added to R primers
  source 1..18: mol_type = other DNA
tgtaaaacgacggccagt

SEQ ID NO: 81 - DNA, 478 bp, synthetic construct
  misc_feature 1..478: note = PHM13395 reference sequence
  source 1..478: mol_type = other DNA
aagtatcgggaaagtcccagtcacaaaatccggcgggtccgcggtggcgcccggacgcaaggaaaagacggagatcggggaggtctccaccgagacgtccgcggcggtgcgcaagaggagaaaggccgacggcagcagctcccctggcactccggtttctacgacggatatgcactgccctcagtgcggcacccatctcatgctaacactgaacatggcggagtccaaatcggagacggggctcgcgaaggacgagtcggccaccgccgcgcctgatcaaggcgggacgggtgagtcttcacagaagaatgttcgggttcggttccatcagttcctgtgagatccagggttccttcctgcccagacaaatcctgggaaacagagccatggtttctcgtctgttatttggaagaacgaaataagaagattttagattaagaattcgttagaataaccttaattttaattaaatagtgaa

SEQ ID NO: 82 - DNA, 589 bp, synthetic construct
  misc_feature 1..589: note = PHM4677 reference sequence
  source 1..589: mol_type = other DNA
cccagtcacaacgagaagaactagagcaacagcagattcctcagtcgaagcaatctggagtgctgatacagtcacgcaggacacgggaggtgacatcagacacaaagagagatggtcgtttccaaaccggagctcagtatggtgatgaaactgagagtgtgacaagtaagacacaagtccatcaaggattcaacagctcaagtactgaacggagtgaaaggagggatccaagtgtgtaccccagggttgcagtacagcgctcttcgtctaaagctgagcagattgaatctccgatggagagagggaagccacaaggagctgaaatgagaagcaccttatttcgaggaaatgaagaggacacagaaacctcatctggaactccaaaagaaagcacccccaaaacaccccctgcacatgttcatcccaagcttccaacagactatgattctttcgccgcacattttaggtctcttcgaacaaaccggccttaggtttacacgacatatagagtttggagtttcagttgaattaagtcatatatacgatactatgatacgttttatggagtgattattactaacgttattaa

SEQ ID NO: 83 - DNA, 651 bp, synthetic construct
  misc_feature 1..651: note = PHM3418 reference sequence
  source 1..651: mol_type = other DNA
gasggatggaagatgctacatatctacagggggttttctcacacaagactcactcttgaatattaaatgtccagtcagtattgttcttcagaatctgaaatcttaataagtacagatatacacggagaattgggtgaattcacccgggcaacaagaagacaactcgtggcaggcttttgtgtacatacctcctcaagacagatgggaagtcttgaaggtaaattatcgttttctatcgatcaacatccagagtatgtgactttttttagtgatgaagaaaccgttcccattccatacagatccctcttgatcgctatttacccacatggagaggaaatgtgatccaggcaaagttggaaatgaaccctgctcggatcgtggggatgtctctctctgtaaacgcagaaggcggtgttcctggcgccaagactgggcctggtgattttaggcttgatgttgcttggatcaaagcgttgagagctttgtgaactccacaagtcatagttttatttcacatcggccctttccttctttatcaccctgctccagtggcgccgctgaactcatcagccgaccacaaccacaggagtaaccatagcacagattgccaactcctttatgcacttaataatgattttttaatatctwttt

SEQ ID NO: 84 - DNA, 703 bp, synthetic construct
  misc_feature 1..703: note = PHM15992 reference sequence
  source 1..703: mol_type = other DNA
attttttggaagctgaacaatttccatgaagaaggtactcttgttttttagatattggagcgaggcatttaccatccaaagatggggttcttgctttcttaaagaaaaaaaagtagctgtaagctgatttaccaggttgaccctagttagatatcttaaatttgaaatatatgctgtggctttattgtgaggtaataatatttttctcagccatgttagttacatccaagaattgggctgtttactaagtttcttgtttttttgttgtaccagaagtgaaatcctagattaatacatggaggtcatgaaacaattaatagaaaatgctacttttttgtactaacatttgtttctcttgtgagcaggccttgtatgagacattgattcggcaggatgagctgcttgcatatattgaccaacaacagacagccaaattttgtgtaagttacagccgttcgtatagtttgccttttcctttcaagaacatatcatcttaatgcttccctcttctagtcaagggtaccaaatacgcaatttcttatttgtccattcatcatttgcagcggcagaagttctgtttctaagtactggagtacctgccacctattttcgtctctttggagatcgcatgcagctattgtggacccagtatacttgcaaatgttttcatatttgttgcagttatggataattgggaaaaacc

SEQ ID NO: 85 - DNA, 466 bp, synthetic construct
  misc_feature 1..466: note = PHM2817 reference sequence
  source 1..466: mol_type = other DNA
aagggttaggagaagatcccagtcaaaacgatatttacagtttcggagtggtgctgttagaatgtgcgaccgctagggatccagtcgattactctaagcctgcagatgaggtacgagttctccctgtttcagacaattggtgtgattgtatttccatttacttcttaaacctcttctattgtttgtttcaggtgaatctcatagagtggcttaaaatgatggtccactcaccagtaagagggcagaggaggtagtggatccaaacctcaatgttaagccaccaaaacgtgccctcaagcggacaatcctggttggcttcaagtgtgtcgatcctgacgctgacaagaggccaaagatgagtcacgttgtccagatgcttgaagcagttcagaatgcatatcatgaagtactcatctcatcctaacattttctttctcgtgctctgctttttatcgcacaaaaaaaa

SEQ ID NO: 86 - DNA, 486 bp, synthetic construct
  misc_feature 1..486: note = PHM7446 reference sequence
  source 1..486: mol_type = other DNA
aaaaaaaaccaaatacaaaatggctaaagatgcgggaagtcccagtcaaaacgtggcttacagctgctctgcttcagcttgctcctgataaacagtacttgctgcctagttcatcaactagtacaagtttgaaccatggtttgctggttggttcctttcctgataggggtatagggaggtcgtcagcagttgagcataaatgtaacctggcaggcacgtcttatggggaaggaactgttgaacacacagaaaatggtcatgtgttatcaaccagttctgtcaaaggaaatgagggaactaaaaacagaaaagcggacaatgaaatgatctggcaagctgtgcttgagagtatccaatcagatacattgagaaaaatgatggctaaagaggccaggctaaactctgtcagcctaggaacaggtaagattctcaatctgtcatccatatcagttttacaatcatcagaatttccaactttgctgtaaa

SEQ ID NO: 87 - DNA, 707 bp, synthetic construct
  misc_feature 1..707: note = NLB17_A reference sequence
  source 1..707: mol_type = other DNA
gcatatgggcctgcctgttcgcataagtacaccctccgtctaaaaagaataaaaatctcatttcttgatgagtcaaaaagttcaaatttaagaaaatatatgttatgacacgaatatttataatgcgtaataagtactgctaaattaattttaaaataaaattttcataataaacctatttgaagatacaagtattggtactatttctaataaatctaatcaaactggtgttatatcttttgtaacaaatttgtgctttatgtttctggtgacgtgaatcagcttaatcttgctcaaatctaacattgtcttttgttcgttggcatacaggatcaaaaagaaaagaagcagcacctattgttggtaagagcctatagtcaatacacatgttcatttcgtctaaaagagcagaagaaaagcatgtgatgaattattgccatgtcatgtttaaaatacagaattctcaaaaacaaaaaaaaacttggaatccactaaccactgatagcattgtagaaaatttcatcctcccgttgggcagtacactgatgagtttacatgctgactagtggtgcgcatttgttctttgccaattgagtttttagaatgctttgcagctgaattcacatgtgattttttttgtgatgcaggtgctgttgccgttgcattcctgtgtctagtcattctcacatccttcttggctgtagata

SEQ ID NO: 88 - DNA, 961 bp, synthetic construct
  misc_feature 1..961: note = NLB17_E reference sequence
  source 1..961: mol_type = other DNA
gttctttgccattgagtttttagaatgctttgcagctgaattcacatgtgatttttttttgtgatgcaggtgctgttgccgttgccgttgcattcctgtgtctagtcattctcacatccttcttggcttgtagatatggtttgcttcccttcaaatcgaagaacaaaccagggacaaggattgagtccttcctacagaagaacgagagcatacatccgaaaagatacacctacgcggacgtgaaaagaatgacaaaatccttcgctgtgaagctaggccaaggtgggtttggtgctgtatacaaaggcagcctccacgatggccgacaggtagcagtcaagatgctcaaggacacccaaggtgacggcgaggaattcatgaacgaggtggctagcatcagcaggacttctcatgtcaacgtcgtgacacttctagggttttgcttgcaagggtcgaaaagagcactgatctacgagtacatgcccaatggttcgctcgaaaggtatgccttcaccggtgacatgaacagtgagaatttgctaacctgggaaagactatttgacatagcaattggcacggccagagggctcgaatacctacaccggggatgcaacactcggatcgtgcattttgacatcaagccacacaacatcctgttagaccaggatttctgccctaagatctctgactttggactggccaagctatgtctgaacaaagagagcgctatctccattgttggcgcaagagggacgatagggtatatcgccccggaggtctactcaaagcaatttggaacaataagcagcaagtctgatgtctatagctatgggatgatggtccttgagatggttggagcaagggacaggaatacaagcgcagatagtgaccatagcagccaatatttccctcagtggctttatgagcatttggacgactattgtgttggtgctccgagatt

SEQ ID NO: 89 - DNA, 539 bp, synthetic construct
  misc_feature 1..539: note = NLB17_3 reference sequence
  source 1..539: mol_type = other DNA
cagctatgaccatggccgagtcgaaacaagttgagttcatgacgagtcgagcaagctcacaatccacgagtaatttttttccagtcctacctaagactaaagtttagtcctagaactaaattttagtctctatctgtttggttctataaactaaacaggttcagaacaaataaaatacactatagaaaaactgaaatacccttctatgattaaggcgtcactaagcgagagcaataaatgaagggtagagagagaaataaatatgttttagtctcttttagctaccatttgagagagtaaagactaaaatgaaaggtcccttgtaggctttggtgttttggatgacaacacaattaaaggtctaattaagatgttaagtgttgagcaggtacttagtgaaaagcttccaaggctcaacacatggagacaagagtgatataccatatataagctgagttggatatggtctatggatatcaggagtcaaagtgaaagattgtcattgatcaagaatttggatacaagaagcctacttgact

SEQ ID NO: 90 - DNA, 784 bp, synthetic construct
  misc_feature 1..784: note = NL B18_A reference sequence
  source 1..784: mol_type = other DNA
aaagcatatgggcctgcctgttcgcataagtacaccctccgtctaaaaaagaataaaaatctcatttcttgatgagtcaaaaaagttcaaatttaagaaaatatatgttacgacacgaatatttataatgcgtaataagtactgctagattaattctaaaataaaattttcataataaacctatttgaagatacaagtatattggtactatttctaataaatctaatcaaactggtgttatatcttttggaacaaatttgtgctttatgtttctggttgacgtgaatcagcttaatcttgctcaaatctaacattgtcttttgttcgttggcatacaggatcaacaaaaaggaaagaagcagcatctattgttggtaagagcctatagtcaataatacccatgttcatttcgtctaaaagagcagaagaaaagcatatgatgaattattgccatgtcttgtttaaaatacagaattctcaaaaacaaaaacaaaaaaaaacttggaatccactaaccagtaaccactgatagcattgtagaaaatttcatcctccctttgggcaatacacactgatgagtttacatgctgactagtggtgcgcatttgttcttttgccaattgaatttttagaatgctttgcagctgaattcacttgtggtgttttttttttgtgtgatgcaggtgctgttgttgccgttgcattcctgtgtctagtcattctcacatgcttcttggcttgtagacatggttcgctgcccttcaaatcgaagaacaaactggcc

SEQ ID NO: 91 - DNA, 624 bp, synthetic construct
  misc_feature 1..624: note = NLB18_E reference sequence
  source 1..624: mol_type = other DNA
ttaatctcggagcaccaacacaatagtcgtccaaatgctcataaagccactgagggaaatattggctgctatggtcactactatctgcgcttgcgcttgtattcctttcccttgctccaaccatctcaaggaccatcatcccatagctatagacatcagacttgctgctgattgttccaaattgctttgagtagacctccggggcgatataccctatcgtccctcttgcgccaacaatggagatagcgctctctttgttcagacatagcttggccagtccaaagtcagagatcttagggcagaaatcctggtctaacaggatgttgtgtggcttgatgtcaaaatgcacgatccgagtgttgcatccccggtgtaggtattcgagccctctggccgtgtgccaattgctatgtcaaatagtctttcccaggttagcaaattctcactgttcatgtcaccggtgaaggcatacctttcgagcgaaccattgggcatgtactcgtagatcagtgctcttttcgacccttgcaagcaaaaccctagaagtgtcacgacgttgacatgagaagtcctgctgatgctagccacctcgttcatgaattcctcgccgtcaccttgggtgtc

SEQ ID NO: 92 - DNA, 1463 bp, Zea mays
  source 1..1463: mol_type = other DNA
gttggaggcttggagctaacaacgcggcttgatgagggtgaacccagccccacctcgtctaccacgtcttctcctcggcatggctgctcacctaccacgtctccccgtcctcctcctcgtcctcctcgctgcccatgtcgtctccacctccacccgtgccgagcctcctcttccgagcacttacaacgtctccatgttctcggaatcgttctggtgcggcggaatcgagttggaatggaatcggacatgggaggatcagtgtggccagtgcgagggattgggctccggcggacggtgcgcctacagccagaagagagaattcctgggctgcttgtgcagcggagggaaggtgggcaacccgttctgcaaaccatcgacatcgagatcaaaaagaaaagaagcagcacctattgttggtgctgttgccgttgcattcctgtgtctagtcattctcacatccttcttggcttgtagatatggtttgcttcccttcaaatcgaagaacaaaccagggacaaggattgagtccttcctacagaagaacgagagcatacatccgaaaagatacacctacgcggacgtgaaaagaatgacaaaatccttcgctgtgaagctaggccaaggtgggtttggtgctgtatacaaaggcagcctccacgatggccgacaggtagcagtcaagatgctcaaggacacccaaggtgacggcgaggaattcatgaacgaggtggctagcatcagcaggacttctcatgtcaacgtcgtgacacttctagggttttgcttgcaagggtcgaaaagagcactgatctacgagtacatgcccaatggttcgctcgaaaggtatgccttcaccggtgacatgaacagtgagaatttgctaacctgggaaagactatttgacatagcaattggcacggccagagggctcgaatacctacaccggggatgcaacactcggatcgtgcattttgacatcaagccacacaacatcctgttagaccaggatttctgccctaagatctctgactttggactggccaagctatgtctgaacaaagagagcgctatctccattgttggcgcaagagggacgatagggtatatcgccccggaggtctactcaaagcaatttggaacaataagcagcaagtctgatgtctatagctatgggatgatggtccttgagatggttggagcaagggacaggaatacaagcgcagatagtgaccatagcagccaatatttccctcagtggctttatgagcatttggacgactattgtgttggtgcttccgagattaatggtgaaaccacagagctcgtgaggaagatgatagttgtaggtctgtggtgcatacaagtgattccgactgatcgaccaacaatgacgagagtcgtcgagatgttggaagggagcacaagtaatctagagttgccacccagagttcttttgagctgac

SEQ ID NO: 93 - protein, 476 aa, Zea mays
MRVNPAPPRLPRLLLGMAAHLPRLPVLLLVLLAAHVVSTSTRAEPPLPSTYNVSMFSESFWCGGIELEWNRTWEDQCGQCEGLGSGGRCAYSQKREFLGCLCSGGKVGNPFCKPSTSRSKRKEAAPIVGAVAVAFLCLVILTSFLACRYGLLPFKSKNKPGTRIESFLQKNESIHPKRYTYADVKRMTKSFAVKLGQGGFGAVYKGSLHDGRQVAVKMLKDTQGDGEEFMNEVASISRTSHVNVVTLLGFCLQGSKRALIYEYMPNGSLERYAFTGDMNSENLLTWERLFDIAIGTARGLEYLHRGCNTRIVHFDIKPHNILLDQDFCPKISDFGLAKLCLNKESAISIVGARGTIGYIAPEVYSKQFGTISSKSDVYSYGMMVLEMVGARDRNTSADSDHSSQYFPQWLYEHLDDYCVGASEINGETTELVRKMIVVGLWCIQVIPTDRPTMTRVVEMLEGSTSNLELPPRVLLS

SEQ ID NO: 94 - DNA, 2064 bp, Zea mays
  source 1..2064: mol_type = other DNA
tccacctcgtctaccacgtcttctccccgccatggctgctcaccagcctcacctctccgtcctcctcctcgtcctcctcgctgcccatgtcgtctccacctccgcccatggcgagcctcctcttccgagcccttacaacacctccgcccatggcgagcctcctcttccgagcacttacaacgcctccatgtgctcgtcgttctggtgtggcggcgtcgagatccgctacccgttctatcttgccaacgcaatcgccgactacagcgggagctactactcctgcggctacaccgacttgagcgtttcctgcgaactcgaggtcgaggggtcgccgacgacctggacccctaccatccgtctcggcggcggcgactacaccgtcaagaacatctcctacctctacgaccagcagaccatctcactggcggacagagatgtgctcggaggcggcggctgccccgtcgtccgccacaacgtcagcttcgacgagacgtggctgcacctgcacaacgccagcgccttcgacaacctcaccttcttcttcggatgccactgggggccacggaatacaccgcctgaatttgccgactacaacatcagctgcgccgggttcaatactccaactatcagcggtggaaggtccttcgtgttcaagactggagatcttgacgaacaagaggagcaggagttggctttacactgcgacgaggttttctccgtgccagtgagaagagatgctctgcaggcgatcgtcagcaacttcagcctcacacgggacgggtacggcgaggtgcttaggcaggggttcgagttggaatggaatcggacatcggaggatcagtgtggccggtgcgagggatcgggctccggcggatggtgcgcctacagccagaagagagaattcctgggctgcttgtgcagcggagggaaggtgggcagcccgttctgcaaaccatcgagatcaaaaaggaaagaaggacctattgttggtgctgttgccgttgcattcctgtgtctagtcattctcacatgcttcttggcttgtagacatggttcgctgcccttcaaatcggagaacaaaccagggacaaggattgagtccttcctacagaagaacgagagtatacatccgaaaagatacacctacgcggacgtgaaaagaatgacaaaatccttcgctgtgaagctaggccaaggtgggtttggtgctgtatacaaaggcagcctccacgatggccgacaggtagcagtcaagatgctgaaggacacccaaggtgacggcgaggaattcatgaacgaggtggctagcatcagcaggacttctcatgtcaacgtcgtgacacttctagggttttgcttgcaagggtcgaaaagagcactgatctacgagtacatgcccaatggttcgctcgaaaggtatgccttcaccggtgacatgaacagtgagaatttgctaacctgggaaaggctatttgacatagcaattggcacggccagagggctcgaatacctacaccggggatgcaacactcggatcgtgcattttgacatcaagccacacaacatcctgttagaccaggatttctgtcctaagatctctgactttggactggccaagctatgtctgaacaaagagagcgctatctccattgctggcgcaagagggacgatagggtatatcgccccggaggtctactcaaagcaatttggaataataagcagcaagtctgatgtctatagctatgggatgatggtccttgagatggttggagcaagggacaggaatacaagcgcagatagtgaccatagcagccaatatttccctcagtggctttatgaacatttggacgactattgtgttggtgcttccgagattaatggtgagaccacagagctcgtgaggaagatgatagttgtaggtctgtggtgcatacaagtgattccgactgatcgaccaacaatgacgagagtcgtcgagatgttggaagggagcacaagtaatctagagttgccacccagagttctcttgagctgacaaagcgtagatatttttcctatcaaatg

SEQ ID NO: 95 - protein, 667 aa, Zea mays
MAAHQPHLSVLLLVLLAAHVVSTSAHGEPPLPSPYNTSAHGEPPLPSTYNASMCSSFWCGGVEIRYPFYLANAIADYSGSYYSCGYTDLSVSCELEVEGSPTTWTPTIRLGGGDYTVKNISYLYDQQTISLADRDVLGGGGCPVVRHNVSFDETWLHLHNASAFDNLTFFFGCHWGPRNTPPEFADYNISCAGFNTPTISGGRSFVFKTGDLDEQEEQELALHCDEVFSVPVRRDALQAIVSNFSLTRDGYGEVLRQGFELEWNRTSEDQCGRCEGSGSGGWCAYSQKREFLGCLCSGGKVGSPFCKPSRSKRKEGPIVGAVAVAFLCLVILTCFLACRHGSLPFKSENKPGTRIESFLQKNESIHPKRYTYADVKRMTKSFAVKLGQGGFGAVYKGSLHDGRQVAVKMLKDTQGDGEEFMNEVASISRTSHVNVVTLLGFCLQGSKRALIYEYMPNGSLERYAFTGDMNSENLLTWERLFDIAIGTARGLEYLHRGCNTRIVHFDIKPHNILLDQDFCPKISDFGLAKLCLNKESAISIAGARGTIGYIAPEVYSKQFGIISSKSDVYSYGMMVLEMVGARDRNTSADSDHSSQYFPQWLYEHLDDYCVGASEINGETTELVRKMIVVGLWCIQVIPTDRPTMTRVVEMLEGSTSNLELPPRVLLS

SEQ ID NO: 96 - DNA, 2061 bp, Zea mays
  source 1..2061: mol_type = other DNA
tccacctcgtctaccacgtcttctcctcgccatggctgctcacctaccacgcctccccgtcctcctcctcgtcctcctcgctgctcatgtcgtctccacctccgcccatgccgagcctcctcttccgagcccttacagcacctccgcccatggcgagcctcctcttccgagcacttacaacgtctccatgtgctcggaatcgttctggtgcggcggcgtcgaaatccgctacccgttctatcttgccaacgcaaccgccgactacagcgggagctactactcctgcggctacaccgacttgagcgtttcctgcaaactcgaggtcgaggggccgacgacgacatggacccctaccatccgtctcggcggcgacaactacaccgtcaagaacatcttgtacgactatcataccatctcactggcggacagcgatgtgctcggaggcggcgagtgccccgtcgtccaccacaacgtcagcttcgacgagacgtggctgcacaaccccagcgccttcgacaacctcaccttcttcttcggatgccactgggggccacgcgatacactgcctgaatttgccggcaacaacatcagctgcgccgggttcagtactccagctatcagcggtggaggctccttcgtgttcaagcctgaagatcttgacgaacatgcggagcaggagttggcttcacactgcgacgaggttttctccgtgccagtgagaagcgaggctctgcagcaggcgatcgtcagcaacctcagcctcggggacgggtacggcgagctgcttaggcaggggatcgagttggaatggaaacggacatcggaggatcagtgtggccagtgcgaggaatcgggctccggcggacggtgcgcctacagccagaagagagaattccttggctgcttgtgcagcggagggaaggcgggcaacccgttctgcaaaccatcaagatcaaaaaggaaagaagcatctattgttggtgctgttgccgttgcattcctgtgtctagtcattctcacatgcttcttggcttgtagacatggttcgctgcccttcaaatcggagaacaaaccagggacaaggattgagtccttcctacagaagaacgagagtatacatccgaaaagatacacctacacggacgtgaaaagaatgacaaaatccttcgctgtgaagctaggccaaggtgggtttggtgctgtatacaaaggcagcctccacgatggccgacaggtagcagtcaagatgctcaaggacacccaaggtgacggcgaggaattcatgaacgaggtggctagcatcagcaggacttctcatgtcaacgtcgtgacacttctagggttttgcttgcaagggtcgaaaagagcactgatctacgagtacatgcccaatggttcgctcgaaaggtatgccttcaccggtgacatgaacagtgagaatttgctaacctgggaaaggctatttgacatagcaattggcacggccagagggctcgaatacctacaccggggatgcaacactcggatcgtgcattttgacatcaagccacacaacatcctgttagaccaggatttctgtcctaagatctctgactttggactggccaagctatgtctgaacaaagagagcgctatctccattgttggcgcaagagggacgatagggtatatcgccccggaggtctactcaaagcaatttggaacaatcagcagcaagtctgatgtctatagctatgggatgatggtccttgagatggttggagcaagggaaaggaatacaagcgcaagcgcagatagtgaccatagcagccaatatttccctcagtggatttatgaacatttggacgactattgtgttggtgcttccgagattaatggtgagaccacagagctcgtgaggaagatgatagttgtaggtctgtggtgcatacaagtgattccgactgatcgaccaacaatgacgagagtcgtcgagatgttggaagggagcacgagtaatctagagttgccacccagagttctcttgagctgacaaagcgtagatatttttcctatcaaatg

SEQ ID NO: 97 - protein, 666 aa, Zea mays
MAAHLPRLPVLLLVLLAAHVVSTSAHAEPPLPSPYSTSAHGEPPLPSTYNVSMCSESFWCGGVEIRYPFYLANATADYSGSYYSCGYTDLSVSCKLEVEGPTTTWTPTIRLGGDNYTVKNILYDYHTISLADSDVLGGGECPVVHHNVSFDETWLHNPSAFDNLTFFFGCHWGPRDTLPEFAGNNISCAGFSTPAISGGGSFVFKPEDLDEHAEQELASHCDEVFSVPVRSEALQQAIVSNLSLGDGYGELLRQGIELEWKRTSEDQCGQCEESGSGGRCAYSQKREFLGCLCSGGKAGNPFCKPSRSKRKEASIVGAVAVAFLCLVILTCFLACRHGSLPFKSENKPGTRIESFLQKNESIHPKRYTYTDVKRMTKSFAVKLGQGGFGAVYKGSLHDGRQVAVKMLKDTQGDGEEFMNEVASISRTSHVNVVTLLGFCLQGSKRALIYEYMPNGSLERYAFTGDMNSENLLTWERLFDIAIGTARGLEYLHRGCNTRIVHFDIKPHNILLDQDFCPKISDFGLAKLCLNKESAISIVGARGTIGYIAPEVYSKQFGTISSKSDVYSYGMMVLEMVGARERNTSASADSDHSSQYFPQWIYEHLDDYCVGASEINGETTELVRKMIVVGLWCIQVIPTDRPTMTRVVEMLEGSTSNLELPPRVLLS